European Patent Application EP 4 775 992 A2, published July 15, 2026. Title: TREATMENT OF MUCOPOLYSACCHARIDOSIS II WITH RECOMBINANT HUMAN IDURONATE-2-SULFATASE (IDS). Applicant: REGENXBIO Inc. Application US 18/356,961, filed July 21, 2023. The sequence listing filed with the application follows.

SEQUENCE LISTING (45 sequences)

SEQ ID NO: 1 - protein, 550 aa, Homo sapiens
  source 1..550: note = Human IDS amino acid sequence
MPPPRTGRGLLWLGLVLSSVCVALGSETQANSTTDALNVLLIIVDDLRPSLGCYGDKLVRSPNIDQLASHSLLFQNAFAQQAVCAPSRVSFLTGRRPDTTRLYDFNSYWRVHAGNFSTIPQYFKENGYVTMSVGKVFHPGISSNHTDDSPYSWSFPPYHPSSEKYENTKTCRGPDGELHANLLCPVDVLDVPEGTLPDKQSTEQAIQLLEKMKTSASPFFLAVGYHKPHIPFRYPKEFQKLYPLENITLAPDPEVPDGLPPVAYNPWMDIRQREDVQALNISVPYGPIPVDFQRKIRQSYFASVSYLDTQVGRLLSALDDLQLANSTIIAFTSDHGWALGEHGEWAKYSNFDVATHVPLIFYVPGRTASLPEAGEKLFPYLDPFDSASQLMEPGRQSMDLVELVSLFPTLAGLAGLQVPPRCPVPSFHVELCREGKNLLKHFRFRDLEEDPYLPGNPRELIAYSQYPRPSDIPQWNSDKPSLKDIKIMGYSIRTIDYRYTVWVGFNPDEFLANFSDIHAGELYFVDSDPLQDHNMYNDSQGGDLFQLLMP

SEQ ID NO: 2 - protein, 24 aa, synthetic construct
  source 1..24: note = Oligodendrocyte-myelin glycoprotein (hOMG) signal peptide
MEYQILKMSLCLFILLFLTPGILC

SEQ ID NO: 3 - protein, 31 aa, synthetic construct
  source 1..31: note = Cellular repressor of E1A-stimulated genes 2(hCREG2) signal peptide
MSVRRGRRPARPGTRLSWLLCCSALLSPAAG

SEQ ID NO: 4 - protein, 28 aa, synthetic construct
  source 1..28: note = V-set and transmembrane domain containing 2B(hVSTM2B) signal peptide
MEQRNRLGALGYLPPLLLHALLLFVADA

SEQ ID NO: 5 - protein, 29 aa, synthetic construct
  source 1..29: note = Protocadherin alpha-1 (hPCADHA1) signal peptide
MVFSRRGGLGARDLLLWLLLLAAWEVGSG

SEQ ID NO: 6 - protein, 19 aa, synthetic construct
  source 1..19: note = FAM19A1 (TAFA1) signal peptide
MAMVSAMSWVLYLWISACA

SEQ ID NO: 7 - protein, 26 aa, synthetic construct
  source 1..26: note = VEGF-A signal peptide
MNFLLSWVHWSLALLLYLHHAKWSQA

SEQ ID NO: 8 - protein, 29 aa, synthetic construct
  source 1..29: note = Fibulin-1 signal peptide
MERAAPSRRVPLPLLLLGGLALLAAGVDA

SEQ ID NO: 9 - protein, 19 aa, synthetic construct
  REGION 1..19: note = Vitronectin signal peptide
  source 1..19: note = Vitronectin signal peptide
MAPLRPLLILALLAWVALA

SEQ ID NO: 10 - protein, 18 aa, synthetic construct
  source 1..18: note = Complement Factor H signal peptide
MRLLAKIICLMLWAICVA

SEQ ID NO: 11 - protein, 19 aa, synthetic construct
  source 1..19: note = Opticin signal peptide
MRLLAFLSLLALVLQETGT

SEQ ID NO: 12 - protein, 18 aa, synthetic construct
  source 1..18: note = Albumin signal peptide
MKWVTFISLLFLFSSAYS

SEQ ID NO: 13 - protein, 18 aa, synthetic construct
  source 1..18: note = Chymotrypsinogen signal peptide
MAFLWLLSCWALLGTTFG

SEQ ID NO: 14 - protein, 20 aa, synthetic construct
  source 1..20: note = Interleukin-2 signal peptide
MYRMQLLSCIALILALVTNS

SEQ ID NO: 15 - protein, 15 aa, synthetic construct
  source 1..15: note = Trypsinogen-2 signal peptide
MNLLLILTFVAAAVA

SEQ ID NO: 16 - protein, 736 aa, synthetic construct
  source 1..736: note = AAV1
MAADGYLPDWLEDNLSEGIREWWDLKPGAPKPKANQQKQDDGRGLVLPGYKYLGPFNGLDKGEPVNAADAAALEHDKAYDQQLKAGDNPYLRYNHADAEFQERLQEDTSFGGNLGRAVFQAKKRVLEPLGLVEEGAKTAPGKKRPVEQSPQEPDSSSGIGKTGQQPAKKRLNFGQTGDSESVPDPQPLGEPPATPAAVGPTTMASGGGAPMADNNEGADGVGNASGNWHCDSTWLGDRVITTSTRTWALPTYNNHLYKQISSASTGASNDNHYFGYSTPWGYFDFNRFHCHFSPRDWQRLINNNWGFRPKRLNFKLFNIQVKEVTTNDGVTTIANNLTSTVQVFSDSEYQLPYVLGSAHQGCLPPFPADVFMIPQYGYLTLNNGSQAVGRSSFYCLEYFPSQMLRTGNNFTFSYTFEEVPFHSSYAHSQSLDRLMNPLIDQYLYYLNRTQNQSGSAQNKDLLFSRGSPAGMSVQPKNWLPGPCYRQQRVSKTKTDNNNSNFTWTGASKYNLNGRESIINPGTAMASHKDDEDKFFPMSGVMIFGKESAGASNTALDNVMITDEEEIKATNPVATERFGTVAVNFQSSSTDPATGDVHAMGALPGMVWQDRDVYLQGPIWAKIPHTDGHFHPSPLMGGFGLKNPPPQILIKNTPVPANPPAEFSATKFASFITQYSTGQVSVEIEWELQKENSKRWNPEVQYTSNYAKSANVDFTVDNNGLYTEPRPIGTRYLTRPL

SEQ ID NO: 17 - protein, 735 aa, synthetic construct [sequence omitted]

SEQ ID NO: 18 - protein, 736 aa, synthetic construct
  source 1..736: note = AAV3-3
MAADGYLPDWLEDNLSEGIREWWALKPGVPQPKANQQHQDNRRGLVLPGYKYLGPGNGLDKGEPVNEADAAALEHDKAYDQQLKAGDNPYLKYNHADAEFQERLQEDTSFGGNLGRAVFQAKKRILEPLGLVEEAAKTAPGKKGAVDQSPQEPDSSSGVGKSGKQPARKRLNFGQTGDSESVPDPQPLGEPPAAPTSLGSNTMASGGGAPMADNNEGADGVGNSSGNWHCDSQWLGDRVITTSTRTWALPTYNNHLYKQISSQSGASNDNHYFGYSTPWGYFDFNRFHCHFSPRDWQRLINNNWGFRPKKLSFKLFNIQVRGVTQNDGTTTIANNLTSTVQVFTDSEYQLPYVLGSAHQGCLPPFPADVFMVPQYGYLTLNNGSQAVGRSSFYCLEYFPSQMLRTGNNFQFSYTFEDVPFHSSYAHSQSLDRLMNPLIDQYLYYLNRTQGTTSGTTNQSRLLFSQAGPQSMSLQARNWLPGPCYRQQRLSKTANDNNNSNFPWTAASKYHLNGRDSLVNPGPAMASHKDDEEKFFPMHGNLIFGKEGTTASNAELDNVMITDEEEIRTTNPVATEQYGTVANNLQSSNTAPTTGTVNHQGALPGMVWQDRDVYLQGPIWAKIPHTDGHFHPSPLMGGFGLKHPPPQIMIKNTPVPANPPTTFSPAKFASFITQYSTGQVSVEIEWELQKENSKRWNPEIQYTSNYNKSVNVDFTVDTNGVYSEPRPIGTRYLTRNL

SEQ ID NO: 19 - protein, 734 aa, synthetic construct
  source 1..734: note = AAV4-4
MTDGYLPDWLEDNLSEGVREWWALQPGAPKPKANQQHQDNARGLVLPGYKYLGPGNGLDKGEPVNAADAAALEHDKAYDQQLKAGDNPYLKYNHADAEFQQRLQGDTSFGGNLGRAVFQAKKRVLEPLGLVEQAGETAPGKKRPLIESPQQPDSSTGIGKKGKQPAKKKLVFEDETGAGDGPPEGSTSGAMSDDSEMRAAAGGAAVEGGQGADGVGNASGDWHCDSTWSEGHVTTTSTRTWVLPTYNNHLYKRLGESLQSNTYNGFSTPWGYFDFNRFHCHFSPRDWQRLINNNWGMRPKAMRVKIFNIQVKEVTTSNGETTVANNLTSTVQIFADSSYELPYVMDAGQEGSLPPFPNDVFMVPQYGYCGLVTGNTSQQQTDRNAFYCLEYFPSQMLRTGNNFEITYSFEKVPFHSMYAHSQSLDRLMNPLIDQYLWGLQSTTTGTTLNAGTATTNFTKLRPTNFSNFKKNWLPGPSIKQQGFSKTANQNYKIPATGSDSLIKYETHSTLDGRWSALTPGPPMATAGPADSKFSNSQLIFAGPKQNGNTATVPGTLIFTSEEELAATNATDTDMWGNLPGGDQSNSNLPTVDRLTALGAVPGMVWQNRDIYYQGPIWAKIPHTDGHFHPSPLIGGFGLKHPPPQIFIKNTPVPANPATTFSSTPVNSFITQYSTGQVSVQIDWEIQKERSKRWNPEVQFTSNYGQQNSLLWAPDAAGKYTEPRAIGTRYLTHHL

SEQ ID NO: 20 - protein, 724 aa, synthetic construct
  source 1..724: note = AAV5
MSFVDHPPDWLEEVGEGLREFLGLEAGPPKPKPNQQHQDQARGLVLPGYNYLGPGNGLDRGEPVNRADEVAREHDISYNEQLEAGDNPYLKYNHADAEFQEKLADDTSFGGNLGKAVFQAKKRVLEPFGLVEEGAKTAPTGKRIDDHFPKRKKARTEEDSKPSTSSDAEAGPSGSQQLQIPAQPASSLGADTMSAGGGGPLGDNNQGADGVGNASGDWHCDSTWMGDRVVTKSTRTWVLPSYNNHQYREIKSGSVDGSNANAYFGYSTPWGYFDFNRFHSHWSPRDWQRLINNYWGFRPRSLRVKIFNIQVKEVTVQDSTTTIANNLTSTVQVFTDDDYQLPYVVGNGTEGCLPAFPPQVFTLPQYGYATLNRDNTENPTERSSFFCLEYFPSKMLRTGNNFEFTYNFEEVPFHSSFAPSQNLFKLANPLVDQYLYRFVSTNNTGGVQFNKNLAGRYANTYKNWFPGPMGRTQGWNLGSGVNRASVSAFATTNRMELEGASYQVPPQPNGMTNNLQGSNTYALENTMIFNSQPANPGTTATYLEGNMLITSESETQPVNRVAYNVGGQMATNNQSSTTAPATGTYNLQEIVPGSVWMERDVYLQGPIWAKIPETGAHFHPSPAMGGFGLKHPPPMMLIKNTPVPGNITSFSDVPVSSFITQYSTGQVTVEMEWELKKENSKRWNPEIQYTNNYNDPQFVDFAPDSTGEYRTTRPIGTRYLTRPL

SEQ ID NO: 21 - protein, 736 aa, synthetic construct
  source 1..736: note = AAV6
MAADGYLPDWLEDNLSEGIREWWDLKPGAPKPKANQQKQDDGRGLVLPGYKYLGPFNGLDKGEPVNAADAAALEHDKAYDQQLKAGDNPYLRYNHADAEFQERLQEDTSFGGNLGRAVFQAKKRVLEPFGLVEEGAKTAPGKKRPVEQSPQEPDSSSGIGKTGQQPAKKRLNFGQTGDSESVPDPQPLGEPPATPAAVGPTTMASGGGAPMADNNEGADGVGNASGNWHCDSTWLGDRVITTSTRTWALPTYNNHLYKQISSASTGASNDNHYFGYSTPWGYFDFNRFHCHFSPRDWQRLINNNWGFRPKRLNFKLFNIQVKEVTTNDGVTTIANNLTSTVQVFSDSEYQLPYVLGSAHQGCLPPFPADVFMIPQYGYLTLNNGSQAVGRSSFYCLEYFPSQMLRTGNNFTFSYTFEDVPFHSSYAHSQSLDRLMNPLIDQYLYYLNRTQNQSGSAQNKDLLFSRGSPAGMSVQPKNWLPGPCYRQQRVSKTKTDNNNSNFTWTGASKYNLNGRESIINPGTAMASHKDDKDKFFPMSGVMIFGKESAGASNTALDNVMITDEEEIKATNPVATERFGTVAVNLQSSSTDPATGDVHVMGALPGMVWQDRDVYLQGPIWAKIPHTDGHFHPSPLMGGFGLKHPPPQILIKNTPVPANPPAEFSATKFASFITQYSTGQVSVEIEWELQKENSKRWNPEVQYTSNYAKSANVDFTVDNNGLYTEPRPIGTRYLTRPL

SEQ ID NO: 22 - protein, 737 aa, synthetic construct
  source 1..737: note = AAV7
MAADGYLPDWLEDNLSEGIREWWDLKPGAPKPKANQQKQDNGRGLVLPGYKYLGPFNGLDKGEPVNAADAAALEHDKAYDQQLKAGDNPYLRYNHADAEFQERLQEDTSFGGNLGRAVFQAKKRVLEPLGLVEEGAKTAPAKKRPVEPSPQRSPDSSTGIGKKGQQPARKRLNFGQTGDSESVPDPQPLGEPPAAPSSVGSGTVAAGGGAPMADNNEGADGVGNASGNWHCDSTWLGDRVITTSTRTWALPTYNNHLYKQISSETAGSTNDNTYFGYSTPWGYFDFNRFHCHFSPRDWQRLINNNWGFRPKKLRFKLFNIQVKEVTTNDGVTTIANNLTSTIQVFSDSEYQLPYVLGSAHQGCLPPFPADVFMIPQYGYLTLNNGSQSVGRSSFYCLEYFPSQMLRTGNNFEFSYSFEDVPFHSSYAHSQSLDRLMNPLIDQYLYYLARTQSNPGGTAGNRELQFYQGGPSTMAEQAKNWLPGPCFRQQRVSKTLDQNNNSNFAWTGATKYHLNGRNSLVNPGVAMATHKDDEDRFFPSSGVLIFGKTGATNKTTLENVLMTNEEEIRPTNPVATEEYGIVSSNLQAANTAAQTQVVNNQGALPGMVWQNRDVYLQGPIWAKIPHTDGNFHPSPLMGGFGLKHPPPQILIKNTPVPANPPEVFTPAKFASFITQYSTGQVSVEIEWELQKENSKRWNPEIQYTSNFEKQTGVDFAVDSQGVYSEPRPIGTRYLTRNL

SEQ ID NO: 23 - protein, 738 aa, synthetic construct
  source 1..738: note = AAV8
MAADGYLPDWLEDNLSEGIREWWALKPGAPKPKANQQKQDDGRGLVLPGYKYLGPFNGLDKGEPVNAADAAALEHDKAYDQQLQAGDNPYLRYNHADAEFQERLQEDTSFGGNLGRAVFQAKKRVLEPLGLVEEGAKTAPGKKRPVEPSPQRSPDSSTGIGKKGQQPARKRLNFGQTGDSESVPDPQPLGEPPAAPSGVGPNTMAAGGGAPMADNNEGADGVGSSSGNWHCDSTWLGDRVITTSTRTWALPTYNNHLYKQISNGTSGGATNDNTYFGYSTPWGYFDFNRFHCHFSPRDWQRLINNNWGFRPKRLSFKLFNIQVKEVTQNEGTKTIANNLTSTIQVFTDSEYQLPYVLGSAHQGCLPPFPADVFMIPQYGYLTLNNGSQAVGRSSFYCLEYFPSQMLRTGNNFQFTYTFEDVPFHSSYAHSQSLDRLMNPLIDQYLYYLSRTQTTGGTANTQTLGFSQGGPNTMANQAKNWLPGPCYRQQRVSTTTGQNNNSNFAWTAGTKYHLNGRNSLANPGIAMATHKDDEERFFPSNGILIFGKQNAARDNADYSDVMLTSEEEIKTTNPVATEEYGIVADNLQQQNTAPQIGTVNSQGALPGMVWQNRDVYLQGPIWAKIPHTDGNFHPSPLMGGFGLKHPPPQILIKNTPVPADPPTTFNQSKLNSFITQYSTGQVSVEIEWELQKENSKRWNPEIQYTSNYYKSTSVDFAVNTEGVYSEPRPIGTRYLTRNL

SEQ ID NO: 24 - protein, 736 aa, synthetic construct
  source 1..736: note = hu31
MAADGYLPDWLEDTLSEGIRQWWKLKPGPPPPKPAERHKDDSRGLVLPGYKYLGPGNGLDKGEPVNAADAAALEHDKAYDQQLKAGDNPYLKYNHADAEFQERLKEDTSFGGNLGRAVFQAKKRLLEPLGLVEEAAKTAPGKKRPVEQSPQEPDSSAGIGKSGSQPAKKKLNFGQTGDTESVPDPQPIGEPPAAPSGVGSLTMASGGGAPVADNNEGADGVGSSSGNWHCDSQWLGDRVITTSTRTWALPTYNNHLYKQISNSTSGGSSNDNAYFGYSTPWGYFDFNRFHCHFSPRDWQRLINNNWGFRPKRLNFKLFNIQVKEVTDNNGVKTIANNLTSTVQVFTDSDYQLPYVLGSAHEGCLPPFPADVFMIPQYGYLTLNDGGQAVGRSSFYCLEYFPSQMLRTGNNFQFSYEFENVPFHSSYAHSQSLDRLMNPLIDQYLYYLSKTINGSGQNQQTLKFSVAGPSNMAVQGRNYIPGPSYRQQRVSTTVTQNNNSEFAWPGASSWALNGRNSLMNPGPAMASHKEGEDRFFPLSGSLIFGKQGTGRDNVDADKVMITNEEEIKTTNPVATESYGQVATNHQSAQAQAQTGWVQNQGILPGMVWQDRDVYLQGPIWAKIPHTDGNFHPSPLMGGFGMKHPPPQILIKNTPVPADPPTAFNKDKLNSFITQYSTGQVSVEIEWELQKENSKRWNPEIQYTSNYYKSNNVEFAVSTEGVYSEPRPIGTRYLTRNL

SEQ ID NO: 25 - protein, 736 aa, synthetic construct
  source 1..736: note = hu32
MAADGYLPDWLEDTLSEGIRQWWKLKPGPPPPKPAERHKDDSRGLVLPGYKYLGPGNGLDKGEPVNAADAAALEHDKAYDQQLKAGDNPYLKYNHADAEFQERLKEDTSFGGNLGRAVFQAKKRLLEPLGLVEEAAKTAPGKKRPVEQSPQEPDSSAGIGKSGSQPAKKKLNFGQTGDTESVPDPQPIGEPPAAPSGVGSLTMASGGGAPVADNNEGADGVGSSSGNWHCDSQWLGDRVITTSTRTWALPTYNNHLYKQISNSTSGGSSNDNAYFGYSTPWGYFDFNRFHCHFSPRDWQRLINNNWGFRPKRLNFKLFNIQVKEVTDNNGVKTIANNLTSTVQVFTDSDYQLPYVLGSAHEGCLPPFPADVFMIPQYGYLTLNDGSQAVGRSSFYCLEYFPSQMLRTGNNFQFSYEFENVPFHSSYAHSQSLDRLMNPLIDQYLYYLSKTINGSGQNQQTLKFSVAGPSNMAVQGRNYIPGPSYRQQRVSTTVTQNNNSEFAWPGASSWALNGRNSLMNPGPAMASHKEGEDRFFPLSGSLIFGKQGTGRDNVDADKVMITNEEEIKTTNPVATESYGQVATNHQSAQAQAQTGWVQNQGILPGMVWQDRDVYLQGPIWAKIPHTDGNFHPSPLMGGFGMKHPPPQILIKNTPVPADPPTAFNKDKLNSFITQYSTGQVSVEIEWELQKENSKRWNPEIQYTSNYYKSNNVEFAVNTEGVYSEPRPIGTRYLTRNL

SEQ ID NO: 26 - protein, 736 aa, synthetic construct
  source 1..736: note = AAV9
MAADGYLPDWLEDNLSEGIREWWALKPGAPQPKANQQHQDNARGLVLPGYKYLGPGNGLDKGEPVNAADAAALEHDKAYDQQLKAGDNPYLKYNHADAEFQERLKEDTSFGGNLGRAVFQAKKRLLEPLGLVEEAAKTAPGKKRPVEQSPQEPDSSAGIGKSGAQPAKKRLNFGQTGDTESVPDPQPIGEPPAAPSGVGSLTMASGGGAPVADNNEGADGVGSSSGNWHCDSQWLGDRVITTSTRTWALPTYNNHLYKQISNSTSGGSSNDNAYFGYSTPWGYFDFNRFHCHFSPRDWQRLINNNWGFRPKRLNFKLFNIQVKEVTDNNGVKTIANNLTSTVQVFTDSDYQLPYVLGSAHEGCLPPFPADVFMIPQYGYLTLNDGSQAVGRSSFYCLEYFPSQMLRTGNNFQFSYEFENVPFHSSYAHSQSLDRLMNPLIDQYLYYLSKTINGSGQNQQTLKFSVAGPSNMAVQGRNYIPGPSYRQQRVSTTVTQNNNSEFAWPGASSWALNGRNSLMNPGPAMASHKEGEDRFFPLSGSLIFGKQGTGRDNVDADKVMITNEEEIKTTNPVATESYGQVATNHQSAQAQAQTGWVQNQGILPGMVWQDRDVYLQGPIWAKIPHTDGNFHPSPLMGGFGMKHPPPQILIKNTPVPADPPTAFNKDKLNSFITQYSTGQVSVEIEWELQKENSKRWNPEIQYTSNYYKSNNVEFAVNTEGVYSEPRPIGTRYLTRNL

SEQ ID NO: 27 - protein, 550 aa, Homo sapiens; identical to SEQ ID NO: 1
  source 1..550: note = SP/P22304/IDS_human

SEQ ID NO: 28 - protein, 550 aa, Pan troglodytes
  REGION 1..550: note = TR/K6ZGI9_PANTR
  source 1..550: note = Chimpanzee; note = TR/K6ZGI9_PANTR
MPPPRTGRGLPWLGLVLSSVCVALGSETQANSTTDALNVLLIIVDDLRPSLGCYGDKLVRSPNIDQLASHSLLFQNAFAQQAVCAPSRVSFLTGRRPDPTRLYDFNSYWRVHAGNFSTIPQYFKENGYVTMSVGKVFHPGISSNHTDDSPYSWSFPPYHPSSEKYENTKTCRGPDGELHANLLCPVDVLDVPEGTLPDKQSTEQAIQLLEKMKTSASPFFLAVGYHKPHIPFRYPKEFQKLYPLENITLAPDPEVPDGLPPVAYNPWMDIRQREDVQALNISVPYGPIPVDFQRKIRQSYFASVSYLDTQVGRLLSALDDLQLANSTIIAFTSDHGWALGEHGEWAKYSNFDVATHVPLMFYVPGRTASLPEAGEKLFPYLDPFDSASQLMEPGRQSMDLVELVSLFPTLAGLAGLQAPPRCPVPSFHVELCREGKNLLKHFRFRDLEEDPYLPGNPRELIAYSQYPRPSDIPQWNSDKPSLKDIKIMGYSIRTIDYRYTVWIGFNPDEFLANFSDIHAGELYFVDSDPLQDHNMYNDSQGGDLFQLLMP

SEQ ID NO: 29 - protein, 550 aa, Pan troglodytes
  source 1..550: note = Chimpanzee; note = TR/K7BKV4_PANTR
MPPPRTGRGLPWLGLVLSSVCVALGSETQANSTTDALNVLLIIVDDLRPSLGCYGDKLVRSPNIDQLASHSLLFQNAFAQQAVCAPSRVSFLTGRRPDTTRLYDFNSYWRVHAGNFSTIPQYFKENGYVTMSVGKVFHPGISSNHTDDSPYSWSFPPYHPSSEKYENTKTCRGPDGELHANLLCPVDVLDVPEGTLPDKQSTEQAIQLLEKMKTSASPFFLAVGYHKPHIPFRYPKEFQKLYPLENITLAPDPEVPDGLPPVAYNPWMDIRQREDVQALNISVPYGPIPVDFQRKIRQSYFASVSYLDTQVGRLLSALDDLQLANSTIIAFTSDHGWALGEHGEWAKYSNFDVATHVPLMFYVPGRTASLPEAGEKLFPYLDPFDSASQLMEPGRQSMDLVELVSLFPTLAGLAGLQAPPRCPVPSFHVELCREGKNLLKHFRFRDLEEDPYLPGNPRELIAYSQYPRPSDIPQWNSDKPSLKDIKIMGYSIRTIDYRYTVWIGFNPDEFLANFSDIHAGELYFVDSDPLQDHNMYNDSQGGDLFQLLMP

SEQ ID NO: 30 - protein, 550 aa, Macaca mulatta
  source 1..550: note = TR/H9FTX2_MACMU; note = Rhesus macaque
MPTPGSGRGFLWLGLVLSSVCVALGCETQANSTTDALNILLIIVDDLRPSLGCYGDKLVRSPNIDQLASHSLLFQNAFAQQAVCAPSRVSFLTGRRPDTTRLYDFNSYWRVHAGNFSTIPQYFKENGYVTMSVGKVFHPGITSNHTDDSPYSWSFPPYHPSSEKYENTKTCRGPDGELHANLLCPVDVVDVPEGTLPDKQSTEQAIQLLEKMKTSASPFFLAVGYHKPHIPFRYPKEFQKLYPLENITLAPDSEVPDGLPPVAYNPWMDIRQREDVQALNISVPYGPIPVEFQRKIRQSYFASVSYLDTQVGRLLSALDDLQLANSTIVAFTSDHGWALGEHGEWAKYSNFDVATHVPLMFYVPGRTASLPEAGEKLFPYLDPFDSASELMEPGRQSMDLVELVSLFPTLAGLAGLQVPPRCPVPSFHVELCREGKNLLKHFRFRDLEEDPYLPGNPRELIAYSQYPRPADFPQWNSDKPSLKDIKIMGYSIRTIDYRYTVWVGFNPDEFLANFSDIHAGELYFVDSDPLQDHNMYNDSQGGDLFQLLMP

SEQ ID NO: 31 - protein, 550 aa, Callithrix jacchus
  REGION 1..550: note = TRF7EJG2_CALJA
  source 1..550: note = TRF7EJG2_CALJA; note = White-tufted-ear marmoset
MPPPRTSRCLLLLGLVLGSVCVTLGSQAQASSTTDALNVLLIIVDDLRPSLGCYGDKLVRSPNIDQLASHSLLFQNAFAQQAVCAPSRVSFLTGRRPDTTRLYDFNSYWRVHAGNFSTIPQYFKDNGYVTMSVGKVFHPGISSNHSDDSPYSWSFPPYHPSSEKYENTKTCRGPDGELHANLLCPVDVVDVPEGTLPDKQSTEEAIRLLEKMKTSASPFFLAVGYHKPHIPFRYPKEFQKLYPLENITLAPDPEVPDGLPPVAYNPWMDIRQREDVQALNISVPYGPIPVDFQRKIRQSYFASVSYLDTQVGHLLSALDDLQLANSTIVAFTSDHGWALGEHGEWAKYSNFDVATRVPLMFYVPGRTASLPEADEKLFPYVDPFHSASELMEPGRQSMDLVELVSLFPTLAGLAGLQVPPRCPVPSFHVELCREGKSLLKHFRFHGLEEDPYLPGNPRELIAYSQYPRPADFPQWNSDKPSLKYIKIMGYSIRTVDYRYTVWVGFNPDEFLANFSDIHAGELYFVDSDPLQDHNMYNDSQGGELFQSLMP

SEQ ID NO: 32 - protein, 550 aa, Callithrix jacchus
  source 1..550: note = TR/U3DTL8_CALJA; note = White-tufted-ear marmoset
MPPPRPSRCLLLLGLVLGSVCVTLGSQAQASSTTDALNVLLIIVDDLRPSLGCYGDKLVRSPNIDQLASHSLLFQNAFAQQAVCAPSRVSFLTGRRPDTTRLYDFNSYWRVHAGNFSTIPQYFKDNGYVTMSVGKVFHPGISSNHSDDSPYSWSFPPYHPSSEKYENTKTCRGPDGELHANLLCPVDVVDVPEGTLPDKQSTEEAIRLLEKMKTSASPFFLAVGYHKPHIPFRYPKEFQKLYPLENITLAPDPEVPDGLPPVAYNPWMDIRQREDVQALNISVPYGPIPVDFQRKIRQSYFASVSYLDTQVGHLLSALDDLQLANSTIVAFTSDHGWALGEHGEWAKYSNFDVATRVPLMFYVPGRTASLPEADEKLFPYVDPFHSASELMEPGRQSMDLVELVSLFPTLAGLAGLQVPPRCPVPSFHVELCREGKSLLKHFRFHGLEEDPYLPGNPRELIAYSQYPRPADFPQWNSDKPSLKYIKIMGYSIRTVDYRYTVWVGFNPDEFLANFSDIHAGELYFVDSDPLQDHNMYNDSQGGELFQSLMP

SEQ ID NO: 33 - protein, 550 aa, Macaca mulatta
  source 1..550: note = Rhesus macaque; note = TR/G7NRX7_MACMU
MPTPGSGRGFLWLGLVLSSVCVALGCETQANSTTDALNILLIIVDDLRPSLGCYGDKLVRSPNIDQLASHSLLFQNAFAQQAVCAPSRVSFLTGRRPDTTRLYDFNSYWRVHAGNFSTIPQYFKENGYVTMSVGKVFHPGITSNHTDDSPYSWSFPPYHPSSEKYENTKTCRGPDGELHANLLCPVDVVDVPEGTLPDKQSTEQAIQLLEKMKTSASPFFLAVGYHKPHIPFRYPKEFQKLYPLENITLAPDSEVPDGLPPVAYNPWMDIRQREDVQALNISVPYGPIPVEFQRKIRQSYFASVSYLDTQVGRLLSALDDLQLANSTIVAFTSDHGWALGEHGEWAKYSNFDVATHVPLMFYVPGRTASLPEAGEKLFPYLDPFDSASELMEPGRQSMDLVELVSLFPTLAGLAGLQVPPRCPVPSFHVELCREGKNLLKHFRFRDLEEDPYLPGNPRELIAYSQYPRPADFPQWNSDKPSLKDIKIMGYSIRTIDYRYTVWVGFNPDEFLANFSDIHAGELYFVDSDPLQDHNMYNDSQGGDLLQLLMP

SEQ ID NO: 34 - protein, 550 aa, Macaca fascicularis
  source 1..550: note = Crab-eating macaque; Cynomologous monkey; note = RT/G7Q1V9_MACFA
MPTPGSGRGFLWLGLVLSSVCVALGCETQANSTTDALNILLIIVDDLRPSLGCYGDKLVRSPNIDQLASHSLLFQNAFAQQAVCAPSRVSFLTGRRPDTTRLYDFNSYWRVHAGNFSTIPQYFKENGYVTMSVGKVFHPGITSNHTDDSPYSWSFPPYHPSSEKYENTKTCRGPDGELHANLLCPVDVVDVPEGTLPDKQSTEQAIQLLEKMKTSASPFFLAVGYHKPHIPFRYPKEFQKLYPLENITLAPDSEVPDGLPPVAYNPWMDIRQREDVQALNISVPYGPIPVEFQRKIRQSYFASVSYLDTQVGHLLSALDDLQLANSTIVAFTSDHGWALGEHGEWAKYSNFDVATHVPLMFYVPGRTASLPEAGEKLFPYLDPFDSASELMEPGRQSMDLVELVSLFPTLAGLAGLQVPPRCPVPSFHVELCREGKNLLKHFRFRDLEEDPYLPGNPRELIAYSQYPRPADFPQWNSDKPSLKDIKIMGYSIRTIDYRYTVWVGFNPDEFLANFSDIHAGELYFVDSDPLQDHNMYNDSQGGDLFQLLMP

SEQ ID NO: 35 - protein, 550 aa, Pongo abelii
  source 1..550: note = TR/H2PX10_PONAB; note = Sumatran orangutan
MPPPRTGRGLLWLGLVLSSVCVALGSETQADSTTDGLNVLLIIVDDLRPSLGCYGDKLVRSPNIDQLASHSLLFQNAFAQQAVCAPSRVSFLTGRRPDTTRLYDFNSYWRVHAGNFSTIPQYFKENGYVTMSVGKVFHPGISSNHTDDSPYSWSFPPYHPSSEKYENTKTCRGPDGELHANLIAKKMCWMFPRAPCCDKQSTEQAIQLLEKMKTSASPFFLAVGYHKPHIPFRYPKEFQKLYPLENITLAPDPEVPDGLPPVAYNPWMDIRQREDVQALNISVPYGPIPVDFQQKIRQSYFASVSYLDTQVGRLLSTLDDLQLANSTIIAFTSDHGWALGEHGEWAKYSNFDVATHVPLMFYVPGRTASLPEAGEKLFPYLDPFDSASELMEPGRQSMDLVELVSLFPTLAGLAGLQVPPRCPVPSFHVELCREGKNLLKHFRFRDLEEDPYLPGNPRELIAYSQYPRPADIPQWNSDKPSLKDIKIMGYSIRTIDYRYTVWVGFNPDEFLANFSDIHAGELYFVDSDPLQDHNMYNDSQGGDLFQLLMP

SEQ ID NO: 36 - protein, 550 aa, Chlorocebus sabaeus
  source 1..550: note = Green monkey; note = TR/A0A0D9R4D1_CHLSB
MPTPGSGRGFLWLGLVLSSVCVALGSETQANSTTDALNILLIIVDDLRPSLGCYGDKLVRSPNIDQLASHSLLFQNAFAQQAVCAPSRVSFLTGRRPDTTRLHNFNSYWRVHAGNFSTIPQYFKENGYVTMSVGKVFHPGITSNHTDDSPYSWSFPPYHPSSEKYENTKTCRGPDGELHANLLCPVDVVDVPEGTLPDKQSTEQAIQLLEKMKTSASPFFLAVGYHKPHIPFRYPKEFQKLYPLENITLAPDSEVPDGLPPVAYNPWMDIRQREDVQALNISVPYGPIPVEFQRKIRQSYFASVSYLDTQVGRLLSALDDLQLANSTIVAFTSDHGWALGEHGEWAKYSNFDVATHVPLMFYVPGRTASLPEAGEKLFPYLDPFDSASELMEPGRQSMDLVELVSLFPTLAGLAGLQVPPRCPVPSFHVELCREGKNLLKHFRFRDLEEDPYLPGNPRELIAYSQYPRPADFPQWNSDKPNLKDIKIMGYSIRTIDYRYTVWVGFNPDEFLANFSDIHAGELYFVDSDPLQDHNMYNDSQGGDLFQLLMP

SEQ ID NO: 37 - protein, 550 aa, Nomascus leucogenys
  VARIANT 24: note = Xaa can be any naturally occurring amino acid
  VARIANT 163..168: note = Xaa can be any naturally occurring amino acid
  source 1..550: note = TR/G1RST8/G1RST8_NOMLE; note = Northern white-cheeked gibbon
MSPPRTGQGLLWLGVVLSSVCVAXVTSPKPPSFVDALNVLLIIVDDLRPSLGCYGDKLVRSPNIDQLASHSLLFQNAFAQQAVCAPSRVSFLTGRRPDTTRLYDFNSYWRVHAGNFSTIPQYFKENGYVTMSVGKVFHPGISSNHTDDSPYSWSFPPYHPSSXXXXXXKTCRGPDGELHANLLCPVDVLDVPEGTLPDKQSTEQAIQLLEKMKTSASPFFLAVGYHKPHIPFRYPKEFQKLYPLENITLAPDPEVPDGLPPVAYNPWMDIRQREDVQALNISVPYGPIPVDFQRKIRQSYFASVSYLDTQVGRLLSALDDLQLANSTIIAFTSDHGWALGEHGEWAKYSNFDVATHVPLMFYVPGRTASLPEAGEKLFPYLDPFDSASELMEPGRQSMDLVELVSLFPTLAGLAGLQVPPRCPVPSFHVELCREGKNLLKHFRFRDLEEDPYLPGNPRELIAYSQYPRPADIPQWNSDKPSLKDIKIMGYSIRTIDYRYTVWVGFSPDEFLANFSDIHAGELYFVDSDPLQDHNMYNDSQGGDLFQLLMP

SEQ ID NO: 38 - protein, 550 aa, Macaca mulatta
  source 1..550: note = UPI0000D9F625; note = Rhesus macaque
MPTPGSGRGFLWLGLVLSSVCVALGCETQANSTTDALNILLIIVDDLRPSLGCYGDKLVRSPNIDQLASHSLLFQNAFAQQAVCAPSRVSFLTGRRPDTTRLYDFNSYWRVHAGNFSTIPQYFKENGYVTMSVGKVFHPGITSNHTDDSPYSWSFPPYHPSSEKYENTKTCRGPDGELHANLLCPVDVVDVPEGTLPDKQSTEQAIQLLEKMKTSASPFFLAVGYHKPHIPFRYPKEFQKLYPLENITLAPDSEVPDGLPPVAYNPWMDIRQREDVQALNISVPYGPIPVEFQRKIRQSYFASVSYLDTQVGHLLSALDDLQLANSTIVAFTSDHGWALGEHGEWAKYSNFDVATHVPLMFYVPGRTASLPEAGEKLFPYLDPFDSASELMEPGRQSMDLVELVSLFPTLAGLAGLQVPPRCPVPSFHVELCREGKNLLKHFRFRDLEEDPYLPGNPRELIAYSQYPRPADFPQWNSDKPSLKDIKIMGYSIRTIDYRYTVWVGFNPDEFLANFSDIHAGELYFVDSDPLQDHNMYNDSQGGDLLQLLMP

SEQ ID NO: 39 - protein, 550 aa, Pan paniscus
  source 1..550: note = Pygmy chimpanzee; Bonobo; note = UPI0000274358B
MPPPRTGRGLLWLGLVLSSVCVALGSETQANSTTDALNVLLIIVDDLRPSLGCYGDKLVRSPNIDQLASHSLLFQNAFAQQAVCAPSRVSFLTGRRPDTTRLYDFNSYWRVHAGNFSTIPQYFKENGYVTMSVGKVFHPGISSNHTDDSPYSWSFPPYHPSSEKYENTKTCRGPDGELHANLLCPVDVLDVPEGTLPDKQSTEQAIRLLEKMKTSASPFFLAVGYHKPHIPFRYPKEFQKLYPLENITLAPDPEVPDGLPPVAYNPWMDIRQREDVQALNISVPYGPIPVDFQRKIRQSYFASVSYLDTQVGRLLSALDDLQLANSTIIAFTSDHGWALGEHGEWAKYSNFDVATHVPLMFYVPGRTASLPEAGEKLFPYLDPFDSASQLMEPGRQSMDLVELVSLFPTLAGLAGLQVPPRCPVPSFHVELCREGKNLLKHFRFRDLEEDPYLPGNPRELIAYSQYPRPSDIPQWNSDKPSLKDIKIMGYSIRTIDYRYTVWVGFNPDEFLANFSDIHAGELYFVDSDPLQDHNMYNDSQGGDLFQLLMP

SEQ ID NO: 40 - protein, 550 aa, Papio Anubis
  source 1..550: note = UPI00027F6FC5; note = Olive baboon
MPTPGSGRGFLWLGLVLSSVCVALGCEMQANSTTDALNILLIIVDDLRPSLGCYGDKLVRSPNIDQLASHSLLFQNAFAQQAVCAPSRVSFLTGRRPDTTRLYDFNSYWRVHAGNFSTIPQYFKENGYVTMSVGKVFHPGITSNHTDDSPYSWSFPPYHPSSEKYENTKTCRGPDGELHANLLCPVDVVDVPEGTLPDKQSTEQAIQLLEKMKTSASPFFLAVGYHKPHIPFRYPKEFQKLYPLENITLAPDSEVPDGLPPVAYNPWMDIRQREDVQALNISVPYGPIPVEFQRKIRQSYFASVSYLDTQVGRLLSALDDLQLANSTIVAFTSDHGWALGEHGEWAKYSNFDVATHVPLMFYVPGRTASLPEAGEKLFPYLDPFDSASELMEPGRQSMDLVELVSLFPTLAGLAGLQVPPRCPVPSFHVELCREGKNLLKHFRFRDLEEDPYLPGNPRELIAYSQYPRPADFPQWNSDKPSLKDIKIMGYSIRTIDYRYTVWVGFNPDEFLANFSDIHAGELYFVDSDPLQDHNMYNDSQGGDLFQLLMP

SEQ ID NO: 41 - protein, 550 aa, Saimiri boliviensis
  source 1..550: note = UPI00027FAE03; note = Bolivian squirrel monkey
MPPPRTGLCLLLLGLVLGSVCVTLGSQAQANSTTDALNVLLIIVDDLRPSLGCYGDKLVRSPNIDQLASHSLLFQNAFVQQAVCAPSRVSFLTGRRPDTTRLYDFNSYWRVHAGNFSTIPQYFKDNGYVTMSVGKVFHPGISSNHSDDSPYSWSFPPYHPSSEKYENTKTCRGPDGELHANLLCPVDVVDVPEGTLPDKQSTEEAIRLLKKMKTSASPFFLAVGYHKPHIPFRYPKEFQKLYPLENITLAPDPEVPDGLPPVAYNPWMDIRQREDVQALNISVPYGPIPVDFQRKIRQSYFASVSYLDTQVGHLLSALDDLHLANSTIVAFTSDHGWALGEHGEWAKYSNFDVATRVPLMFYVPGRTASLPETGEKLFPYVDPFHSASELMEPGRQSTDLVELVSLFPTLAGLAGLQVPPRCPVPSFHIELCREGKNLLKHFRFHGLEEDPYLPGNPRELIAYSQYPRPADFPQQNSDKPSLKYIKIMGYSIRTVDYRYTVWVGFNPDEFLANFSDIHAGELYFVDSDPLQDHNMYNDSQGGELFQSLMP

SEQ ID NO: 42 - protein, 550 aa, Macaca fascicularis
  source 1..550: note = UPI0003ABBF28; note = Crab-eating macaque; Cynomologous monkey
MPTPGSGRGFLWLGLVLSSVCVALGCETQANSTTDALNILLIIVDDLRPSLGCYGDKLVRSPNIDQLASHSLLFQNAFAQEAVCAPSRVSFLTGRRPDTTRLYDFNSYWRVHAGNFSTIPQYFKENGYVTMSVGKVFHPGITSNHTDDSPYSWSFPPYHPSSEKYENTKTCRGPDGELHANLLCPVDVVDVPEGTLPDKQSTEQAIQLLEKMKTSASPFFLAVGYHKPHIPFRYPKEFQKLYPLENITLAPDSEVPDGLPPVAYNPWMDIRQREDVQALNISVPYGPIPVEFQRKIRQSYFASVSYLDTQVGRLLSALDDLQLANSTIVAFTSDHGWALGEHGEWAKYSNFDVATHVPLMFYVPGRTASLPEAGEKLFPYLDPFDSASELMEPGRQSMDLVELVSLFPTLAGLAGLQVPPRCPVPSFHVELCREGKNLLKHFRFRDLEEDPYLPGNPRELIAYSQYPRPADFPQWNSDKPSLKDIKIMGYSIRTIDYRYTVWVGFNPDEFLANFSDIHAGELYFVDSDPLQDHNMYNDSQGGDLFQLLMP

SEQ ID NO: 43 - protein, 550 aa, Rhinopithecus roxellana
  source 1..550: note = UPI000533297F; note = Golden snub-nosed monkey
MPTPASGRGFLWLGLVLSSVCVALGSETQANSTTDALNILLIIVDDLRPSLGCYGDKLVRSPNIDQLASHSLLFQNAFAQQAVCAPSRVSFLTGRRPDTTRLYDFNSYWRVHAGNFSTIPQYFKENGYVTMSVGKVFHPGITSNHTDDSPYSWSFPPYHPSSEKYENTKTCRGPDGELHANLLCPVDVVDVPEGTLPDKQSTEQAVQLLEKMKTSASPFFLAVGYHKPHIPFRYPKEFQKLYPLENITLAPDSEVPDGLPPVAYNPWMDIRQREDVQALNISVPYGPIPVDFQRKIRQSYFASVSYLDTQVGHLLSALDDLQLANSTIVAFTSDHGWALGEHGEWAKYSNFDVATHVPLMFYVPGRTASLPEAGEKLFPYLDPFDSASELMEPGRQSMDLVELVSLFPTLAGLAGLQVPPRCPVPSFHVELCREGKNLLKHFRFRDLEEDPYLPGNPRELIAYSQYPRPADFPQWNSDKPSLKDIKIMGYSIRTIDYRYTVWVGFNPDEFLANFSDIHAGELYFVDSDPFQDHNMYNDSQGGDLFQLLMP

SEQ ID NO: 44 - protein, 550 aa, Colobus angolensis
  source 1..550: note = UPI0005F40BD2; note = Peters Angolan colobus
MPTPASGRGFLWLGLVLRSVCVALGSETQANSTTDALNILLIIVDDLRPSLGCYGDKLVRSPNIDQLASHSLLFQNAFAQQAVCTPSHVSFLTGRRPDTTRLYDFNSYWRVHAGNFSTIPQYFKENGYVTMSVGKVFHPGITSNHTDDSPYSWSFPPYHPSSEKYENTKTCRGPDGELHANLLCPVDVVDVPEGTLPDKQSTEQAIQLLEKMKTSASPFFLAVGYHKPHIPFRYPKEFQKLYPLENITLAPDSEVPDGLPPVAYNPWMDIRQREDVQALNISVPYGPIPVDFQRKIRQSYFASVSYLDTQVGHLLSALDDLQLANSTIVAFTSDHGWALGEHGEWAKYSNFDVATHVPLMFYVPGRTASLPEAGEKLFPYLDPFDSASELMEPGRQSMDLVELVSLFPTLAGLAGLQVPPRCPVPSFHVELCREGKNLLKHFRFRDLEEDPYLPGNPRELIAYSQYPRPADFPQWNSDKPSLKDIKIMGYSIRTIDYRYTVWVGFNPDEFLANFSDIHAGELYFVDSDPLQDHNMYNDSQGGDLFQLLMP

SEQ ID NO: 45 - DNA, 3967 bp, synthetic construct
  source 1..3967: mol_type = other DNA; note = CB7.CI.hIDS.RBG
gctgcgcgctcgctcgctcactgaggccgcccgggcaaagcccgggcgtcgggcgacctttggtcgcccggcctcagtgagcgagcgagcgcgcagagagggagtggccaactccatcactaggggttccttgtagttaatgattaacccgccatgctacttatctaccagggtaatggggatcctctagaactatagctagtcgacattgattattgactagttattaatagtaatcaattacggggtcattagttcatagcccatatatggagttccgcgttacataacttacggtaaatggcccgcctggctgaccgcccaacgacccccgcccattgacgtcaataatgacgtatgttcccatagtaacgccaatagggactttccattgacgtcaatgggtggactatttacggtaaactgcccacttggcagtacatcaagtgtatcatatgccaagtacgccccctattgacgtcaatgacggtaaatggcccgcctggcattatgcccagtacatgaccttatgggactttcctacttggcagtacatctacgtattagtcatcgctattaccatggtcgaggtgagccccacgttctgcttcactctccccatctcccccccctccccacccccaattttgtatttatttattttttaattattttgtgcagcgatgggggcggggggggggggggggcgcgcgccaggcggggcggggcggggcgaggggcggggcggggcgaggcggagaggtgcggcggcagccaatcagagcggcgcgctccgaaagtttccttttatggcgaggcggcggcggcggcggccctataaaaagcgaagcgcgcggcgggcggggagtcgctgcgacgctgccttcgccccgtgccccgctccgccgccgcctcgcgccgcccgccccggctctgactgaccgcgttactcccacaggtgagcgggcgggacggcccttctcctccgggctgtaattagcgcttggtttaatgacggcttgtttcttttctgtggctgcgtgaaagccttgaggggctccgggagggccctttgtgcggggggagcggctcggggggtgcgtgcgtgtgtgtgtgcgtggggagcgccgcgtgcggctccgcgctgcccggcggctgtgagcgctgcgggcgcggcgcggggctttgtgcgctccgcagtgtgcgcgaggggagcgcggccgggggcggtgccccgcggtgcggggggggctgcgaggggaacaaaggctgcgtgcggggtgtgtgcgtgggggggtgagcagggggtgtgggcgcgtcggtcgggctgcaaccccccctgcacccccctccccgagttgctgagcacggcccggcttcgggtgcggggctccgtacggggcgtggcgcggggctcgccgtgccgggcggggggtggcggcaggtgggggtgccgggcggggcggggccgcctcgggccggggagggctcgggggaggggcgcggcggcccccggagcgccggcggctgtcgaggcgcggcgagccgcagccattgccttttatggtaatcgtgcgagagggcgcagggacttcctttgtcccaaatctgtgcggagccgaaatctgggaggcgccgccgcaccccctctagcgggcgcggggcgaagcggtgcggcgccggcaggaaggaaatgggcggggagggccttcgtgcgtcgccgcgccgccgtccccttctccctctccagcctcggggctgtccgcggggggacggctgccttcgggggggacggggcagggcggggttcggcttctggcgtgtgaccggcggctctagagcctctgctaaccatgttcatgccttcttctttttcctacagctcctgggcaacgtgctggttattgtgctgtctcatcattttggcaaagaattcatgccgccaccccggaccggccgaggccttctctggctgggtctggttctgagctccgtctgcgtcgccctcggatccgaaacgcaggccaactcgaccacagatgctctgaacgttcttctcatcatcgtggatgacctgcgcccctccctgggctgttatggggataagctggtgaggtccccaaatattgaccaactggcatcccacagcctcctcttccagaatgcctttgcgcagcaagcagtgtgcgccccgagccgcgtttctttcctcactggcaggagacctgacaccacccgcctgtacgacttcaactcctactggagggtgcacgctggaaacttctccaccatcccccagtacttcaaggagaatggctatgtgaccatgtcggtgggaaaagtctttcaccctgggatatcttctaaccataccgatgattctccgtatagctggtcttttccaccttatcatccttcctctgagaagtatgaaaacactaagacatgtcgagggccagatggagaactccatgccaacctgctttgccctgtggatgtgctggatgttcccgagggcaccttgcctgacaaacagagcactgagcaagccatacagttgttggaaaagatgaaaacgtcagccagtcctttcttcctggccgttgggtatcataagccacacatccccttcagataccccaaggaatttcagaagttgtatcccttggagaacatcaccctggcccccgatcccgaggtccctgatggcctaccccctgtggcctacaacccctggatggacatcaggcaacgggaagacgtccaagccttaaacatcagtgtgccgtatggtccaattcctgtggactttcagcggaaaatccgccagagctactttgcctctgtgtcatatttggatacacaggtcggccgcctcttgagtgctttggacgatcttcagctggccaacagcaccatcattgcatttacctcggatcatgggtgggctctaggtgaacatggagaatgggccaaatacagcaattttgatgttgctacccatgttcccctgatattctatgttcctggaaggacggcttcacttccggaggcaggcgagaagcttttcccttacctcgacccttttgattccgcctcacagttgatggagccaggcaggcaatccatggaccttgtggaacttgtgtctctttttcccacgctggctggacttgcaggactgcaggttccacctcgctgccccgttccttcatttcacgttgagctgtgcagagaaggcaagaaccttctgaagcattttcgattccgtgacttggaagaggatccgtacctccctggtaatccccgtgaactgattgcctatagccagtatccccggccttcagacatccctcagtggaattctgacaagccgagtttaaaagatataaagatcatgggctattccatacgcaccatagactataggtatactgtgtgggttggcttcaatcctgatgaatttctagctaacttttctgacatccatgcaggggaactgtattttgtggattctgacccattgcaggatcacaatatgtataatgattcccaaggtggagatcttttccagttgttgatgccttgactcgaggacggggtgaactacgcctgaggatccgatctttttccctctgccaaaaattatggggacatcatgaagccccttgagcatctgacttctggctaataaaggaaatttattttcattgcaatagtgtgttggaattttttgtgtctctcactcggaagcaattcgttgatctgaatttcgaccacccataatacccattaccctggtagataagtagcatggcgggttaatcattaactacaaggaacccctagtgatggagttggccactccctctctgcgcgctcgctcgctcactgaggccgggcgaccaaaggtcgcccgacgcccgggctttgcccgggcggcctcagtgagcgagcgagcgcgcag